European Patent Application EP 4 375 294 A1, published May 29, 2024. Title: A cell-penetrating degrading antibody that penetrates into the cytosol of cells and degrades to remove a targeted protein, and its uses thereof. Applicant: Ajou University Industry-Academic Cooperation Foundation. Application KR. The sequence listing filed with the application follows.

SEQUENCE LISTING (34 sequences)

SEQ ID NO: 1 - protein, 17 aa, synthetic construct
  REGION 1..17: note = VL-CDR1
KSSQSLLNSRDGKNYLA

SEQ ID NO: 2 - protein, 7 aa, synthetic construct
  REGION 1..7: note = VL-CDR2
WASTRES

SEQ ID NO: 3 - protein, 9 aa, synthetic construct
  REGION 1..9: note = VL-CDR3
QQYWYWMFT

SEQ ID NO: 4 - protein, 9 aa, synthetic construct
  REGION 1..9: note = VL-CDR3
QQYAAAMFT

SEQ ID NO: 5 - protein, 5 aa, synthetic construct
  REGION 1..5: note = VH-CDR1
SYPMH

SEQ ID NO: 6 - protein, 17 aa, synthetic construct
  REGION 1..17: note = VH-CDR2
VVSYDGSYKYYADSVKG

SEQ ID NO: 7 - protein, 17 aa, synthetic construct
  REGION 1..17: note = VH-CDR2
AINPYNDGNYYADSVKG

SEQ ID NO: 8 - protein, 15 aa, synthetic construct
  REGION 1..15: note = VH-CDR3
ATVRGVTKIRGVFDS

SEQ ID NO: 9 - protein, 11 aa, synthetic construct
  REGION 1..11: note = VH-CDR3
GAYKRGYAMDY

SEQ ID NO: 10 - protein, 76 aa, synthetic construct
  REGION 1..76: note = E4B1227-1302
DAPDEFRDPLMDTLMTDPVRLPSGTIMDRSIILRHLLNSPTDPFNRQTLTESMLEPVPELKEQIQAWMREKQNSDH

SEQ ID NO: 11 - protein, 292 aa, synthetic construct
  REGION 1..292: note = IpaH254-545
LADAVTAWFPENKQSDVSQIWHAFEHEEHANTFSAFLDRLSDTVSARNTSGFREQVAAWLEKLSASAELRQQSFAVAADATESCEDRVALTWNNLRKTLLVHQASEGLFDNDTGALLSLGREMFRLEILEDIARDKVRTLHFVDEIEVYLAFQTMLAEKLQLSTAVKEMRFYGVSGVTANDLRTAEAMVRSREENEFTDWFSLWGPWHAVLKRTEADRWAQAEEQKYEMLENEYPQRVADRLKASGLSGDADAEREAGAQVMRETEQQIYRQLTDEVLALRLPENGSQLHHS

SEQ ID NO: 12 - protein, 62 aa, synthetic construct
  REGION 1..62: note = VHL152-213
TLPVYTLKERCLQVVRSLVKPENYRRLDIVRSLYEDLEDHPNVQKDLERLTQERIAHQRMGD

SEQ ID NO: 13 - protein, 114 aa, synthetic construct
  REGION 1..114: note = beta-TrCP142-255
RDFITALPARGLDHIAENILSYLDAKSLCAAELVCKEWYRVTSDGMLWKKLIEKMVRTDSLWRGLAERRGWGQYLFKNKPPDGNAPPNSFYRALYPKIIQDIETIESNWKCGRH

SEQ ID NO: 14 - protein, 208 aa, synthetic construct
  REGION 1..208: note = SPOP167-374
SVNISGQNTMNMVKVPECRLADELGGLWENSRFTDCCLCVAGQEFQAHKAILAARSPVFSAMFEHEMEESKKNRVEINDVEPEVFKEMMCFIYTGKAPNLDKMADDLLAAADKYALERLKVMCEDALCSNLSVENAAEILILADLHSADQLKTQAVDFINYHASDVLETSGWKSMVVSHPHLVAEAYRSLASAQCPFLGPPRKRLKQS

SEQ ID NO: 15 - protein, 54 aa, synthetic construct
  REGION 1..54: note = DDB261-114
QILPPCRSIVRTLHQHKLGRASWPSVQQGLQQSFLHTLDSYRILQKAAPFDRRA

SEQ ID NO: 16 - protein, 45 aa, synthetic construct
  REGION 1..45: note = SOCS2153-198
TKPLYTSAPSLQHLCRLINKCTGAIWGLPLPTRLKDYLEEYKFQV

SEQ ID NO: 17 - protein, 124 aa, synthetic construct
  REGION 1..124: note = inBC0 VH
QVQLVESGGGVVQPGRSLRLSCAASGFTFSSYPMHWVRQAPGKGLEWVAVVSYDGSYKYYADSVKGRLTISRDNSKNTLYLQMNSLRAEDTAVYYCARATVRGVTKIRGVFDSWGRGALVTVSS

SEQ ID NO: 18 - protein, 124 aa, synthetic construct
  REGION 1..124: note = inBC2 VH
QVQLVESGGGVVQPGRSLRLSCAASGFTFSSYPMHWVRQAPGKGLEWVAVVSYDGSYKYYADSVKGRLTISRDNSKNTLYLQMNSLRAEDTAVYYCARATVRGVTKIRGVFDSWGQGTLVTVSS

SEQ ID NO: 19 - protein, 120 aa, synthetic construct
  REGION 1..120: note = inCT VH
EVQLVESGGGLVQPGGSLRLSCAASGYTFTSYVMHWVRQAPGKGLEWVSAINPYNDGNYYADSVKGRFTISRDNSRKTLYLQMNSLRAEDTAVYYCARGAYKRGYAMDYWGQGTTVTVSS

SEQ ID NO: 20 - protein, 114 aa, synthetic construct
  REGION 1..114: note = inBC0 inBC2 inCT VL
DYQLTQSPSSLSASVGDRVTITCKSSQSLLNSRDGKNYLAWYQQKPGKAPKMLIYWASTRESGVPSRFSGSGSGTDFTLTISSLQPEDFATYFCQQYWYWMFTFGQGTKVEIKR

SEQ ID NO: 21 - protein, 114 aa, synthetic construct
  REGION 1..114: note = inBC2-(AAA) VL
DYQLTQSPSSLSASVGDRVTITCKSSQSLLNSRDGKNYLAWYQQKPGKAPKMLIYWASTRESGVPSRFSGSGSGTDFTLTISSLQPEDFATYFCQQYAAAMFTFGQGTKVEIKR

SEQ ID NO: 22 - protein, 62 aa, synthetic construct
  REGION 1..62: note = inBC2-VHL152-213 V181G, D187K
TLPVYTLKERCLQVVRSLVKPENYRRLDIGRSLYEKLEDHPNVQKDLERLTQERIAHQRMGD

SEQ ID NO: 23 - protein, 46 aa, synthetic construct
  REGION 1..46: note = inBC2-SOCS2153-198-1
TKPLYTSAPSLQHLCRLTINKCTGNYRGLPLPTRLKDYLEEYKFQV

SEQ ID NO: 24 - protein, 46 aa, synthetic construct
  REGION 1..46: note = inBC2-SOCS2153-198-2
TKPLRTSADSLQHLCRLTINKCTGAIWGLPLPTRLKDYLEEYKFQD

SEQ ID NO: 25 - protein, 46 aa, synthetic construct
  REGION 1..46: note = inBC2-SOCS2153-198-3
TKPLYTSAPSLQHLCRLTINKCTGAIWGLPLPTRLKDYLEEYKHQD

SEQ ID NO: 26 - protein, 46 aa, synthetic construct
  REGION 1..46: note = inBC2-SOCS2153-198-4
TKPLYTSAPSLQHLCRLTINKCTGNYRGLPLPTRLKDYLEEYKFQD

SEQ ID NO: 27 - protein, 46 aa, synthetic construct
  REGION 1..46: note = inBC2-SOCS2153-198-5
TKPLRTSAPSLQHLCRLTINKCTGNYRGLPLPTRLKDYLEEYKFQD

SEQ ID NO: 28 - protein, 46 aa, synthetic construct
  REGION 1..46: note = inBC2-SOCS2153-198-6
TKPLYTSAPSLQHLCRLTINKCTGNYRGLPLPTRLKDYLEEYKHQD

SEQ ID NO: 29 - protein, 46 aa, synthetic construct
  REGION 1..46: note = inBC2-SOCS2153-198-7
TKPLYTSAPSLQDLCRLTINKCTGNYRGLPLPTRLKDYLEEKKDQD

SEQ ID NO: 30 - protein, 46 aa, synthetic construct
  REGION 1..46: note = inBC2-SOCS2153-198-8
TKPLYTSAPSLKHLCRLTINKCTGNYRGLPLPTRLKDDLEEYKFQD

SEQ ID NO: 31 - protein, 46 aa, synthetic construct
  REGION 1..46: note = inBC2-SOCS2153-198-9
TKPLYTSAPSLQHLMRLTINKCTGNYRGLPLPTRLKDYLEEYKFQD

SEQ ID NO: 32 - protein, 46 aa, synthetic construct
  REGION 1..46: note = inBC2-SOCS2153-198-10
TKPLYTSAPSLQHLCRLTINKMTGNYRGLPLPTRLKDYLEEYKFQD

SEQ ID NO: 33 - protein, 46 aa, synthetic construct
  REGION 1..46: note = inBC2-SOCS2153-198-11
TKPLYTSAPSLQHLCRLTINKQTGNYRGLPLPTRLKDYLEEYKFQD

SEQ ID NO: 34 - protein, 46 aa, synthetic construct
  REGION 1..46: note = inBC2-SOCS2153-198-12
TKPLYTSAPSLKDLCRLTINKCTGNYRGLPLPTRLKDDLEEKKDQD